European Patent Application EP 4 372 003 A1, published May 22, 2024. Title: ANTIBODY COMBINATION AGAINST REGENERATING ISLET-DERIVED PROTEIN 1α AND DETECTION KIT COMPRISING SAME. Applicant: SENBOLL BioTechnology Co., Ltd. The sequence listing filed with the application follows.

SEQUENCE LISTING (26 sequences)

SEQ ID NO: 1 - protein, 7 aa, Mus musculus
TSGMSVG

SEQ ID NO: 2 - protein, 16 aa, Mus musculus
HIWWNDDKFYNPALKS

SEQ ID NO: 3 - protein, 8 aa, Mus musculus
IEEGWFAY

SEQ ID NO: 4 - protein, 118 aa, Mus musculus
QVTLKESGPGILQPSQTLSLTCSFSGFSLSTSGMSVGWIRQPSGKGLEWLAHIWWNDDKFYNPALKSRLTISKDTSKNQIFLKIASVVTADSATYYCARIEEGWFAYWGQGTLVTVST

SEQ ID NO: 5 - protein, 442 aa, Mus musculus
QVTLKESGPGILQPSQTLSLTCSFSGFSLSTSGMSVGWIRQPSGKGLEWLAHIWWNDDKFYNPALKSRLTISKDTSKNQIFLKIASVVTADSATYYCARIEEGWFAYWGQGTLVTVSTAKTTPPSVYPLAPGSAAQTNSMVTLGCLVKGYFPEPVTVTWNSGSLSSGVHTFPAVLQSDLYTLSSSVTVPSSTWPSETVTCNVAHPASSTKVDKKIVPRDCGCKPCICTVPEVSSVFIFPPKPKDVLTITLTPKVTCVVVDISKDDPEVQFSWFVDDVEVHTAQTQPREEQFNSTFRSVSELPIMHQDWLNGKEFKCRVNSAAFPAPIEKTISKTKGRPKAPQVYTIPPPKEQMAKDKVSLTCMITDFFPEDITVEWQWNGQPAENYKNTQPIMDTDGSYFVYSKLNVQKSNWEAGNTFTCSVLHEGLHNHHTEKSLSHSPGK

SEQ ID NO: 6 - protein, 11 aa, Mus musculus
KASQTMSNDVA

SEQ ID NO: 7 - protein, 7 aa, Mus musculus
YASNRYT

SEQ ID NO: 8 - protein, 9 aa, Mus musculus
QQDYSSPLT

SEQ ID NO: 9 - protein, 107 aa, Mus musculus
SIVMTQTPKFLLVSVGDRVTITCKASQTMSNDVAWYQQKPGQSPKLLIYYASNRYTGVPDRFTGSGYGTDFTFTISTVQAEDLAVYFCQQDYSSPLTFGAGTKLELK

SEQ ID NO: 10 - protein, 214 aa, Mus musculus
SIVMTQTPKFLLVSVGDRVTITCKASQTMSNDVAWYQQKPGQSPKLLIYYASNRYTGVPDRFTGSGYGTDFTFTISTVQAEDLAVYFCQQDYSSPLTFGAGTKLELKRADAAPTVSIFPPSSEQLTSGGASVVCFLNNFYPKDINVKWKIDGSERQNGVLNSWTDQDSKDSTYSMSSTLTLTKDEYERHNSYTCEATHKTSTSPIVKSFNRNEC

SEQ ID NO: 11 - protein, 5 aa, Mus musculus
SYMMH

SEQ ID NO: 12 - protein, 17 aa, Mus musculus
YINPSSGYTDYNQKFKD

SEQ ID NO: 13 - protein, 9 aa, Mus musculus
YRYPHYFDY

SEQ ID NO: 14 - protein, 118 aa, Mus musculus
QVQLQQSATELARPGASVKMSCKASGYTFTSYMMHWVKQRPGQGLEWIGYINPSSGYTDYNQKFKDKTTLTADKSSSTAYMQLSSLTSEDSAVYYCARYRYPHYFDYWGQGTTLTVSS

SEQ ID NO: 15 - protein, 442 aa, Mus musculus
QVQLQQSATELARPGASVKMSCKASGYTFTSYMMHWVKQRPGQGLEWIGYINPSSGYTDYNQKFKDKTTLTADKSSSTAYMQLSSLTSEDSAVYYCARYRYPHYFDYWGQGTTLTVSSAKTTPPSVYPLAPGSAAQTNSMVTLGCLVKGYFPEPVTVTWNSGSLSSGVHTFPAVLQSDLYTLSSSVTVPSSTWPSETVTCNVAHPASSTKVDKKIVPRDCGCKPCICTVPEVSSVFIFPPKPKDVLTITLTPKVTCVVVDISKDDPEVQFSWFVDDVEVHTAQTQPREEQFNSTFRSVSELPIMHQDWLNGKEFKCRVNSAAFPAPIEKTISKTKGRPKAPQVYTIPPPKEQMAKDKVSLTCMITDFFPEDITVEWQWNGQPAENYKNTQPIMDTDGSYFVYSKLNVQKSNWEAGNTFTCSVLHEGLHNHHTEKSLSHSPGK

SEQ ID NO: 16 - protein, 10 aa, Mus musculus
SASSSVSYIH

SEQ ID NO: 17 - protein, 7 aa, Mus musculus
DTSKLAS

SEQ ID NO: 18 - protein, 9 aa, Mus musculus
QQWSSNPPT

SEQ ID NO: 19 - protein, 106 aa, Mus musculus
QIVLTQSPAIMSASPGEKVTMTCSASSSVSYIHWYQQKSGTSPKRWIYDTSKLASGVPARFSGSGSGTSYSLTISSMEAEDAAIYYCQQWSSNPPTFGAGTKLELK

SEQ ID NO: 20 - protein, 213 aa, Mus musculus
QIVLTQSPAIMSASPGEKVTMTCSASSSVSYIHWYQQKSGTSPKRWIYDTSKLASGVPARFSGSGSGTSYSLTISSMEAEDAAIYYCQQWSSNPPTFGAGTKLELKRADAAPTVSIFPPSSEQLTSGGASVVCFLNNFYPKDINVKWKIDGSERQNGVLNSWTDQDSKDSTYSMSSTLTLTKDEYERHNSYTCEATHKTSTSPIVKSFNRNEC

SEQ ID NO: 21 - protein, 450 aa, Mus musculus
DVKLVESGGGLVKPGGSLKLSCAASGFTFSSFSMSWFRQTPDKRLEWVATISSGGSSTYYPDSVKGRFTISRDNAKNTLYLQMTSLKSEDTAIFYCRGGYYGNYDPLDYWGQGTSVTVSAAKTTAPSVYPLAPVCGDTTGSSVTLGCLVKGYFPEPVTLTWNSGSLSSGVHTFPAVLQSDLYTLSSSVTVTSSTWPSQSITCNVAHPASSTKVDKKIEPRGPTIKPCPPCKCPAPNLLGGPSVFIFPPKIKDVLMISLSPIVTCVVVDVSEDDPDVQISWFVNNVEVHTAQTQTHREDYNSTLRVVSALPIQHQDWMSGKEFKCKVNNKDLPAPIERTISKPKGSVRAPQVYVLPPPEEEMTKKQVTLTCMVTDFMPEDIYVEWTNNGKTELNYKNTEPVLDSDGSYFMYSKLRVEKKNWVERNSYSCSVVHEGLHNHHTTKSFSRTPGK

SEQ ID NO: 22 - protein, 214 aa, Mus musculus
DIVMIQSQKFMSTSVGDRVSITCTASHNVDSNVAWYQQKPGQSPQALIYSASYRYSGVPDRFTGSGSGTDFTLTINNVQSEDLAEYFCQQYNSYPLTFGGGTRLEIKRADAAPTVSIFPPSSEQLTSGGASVVCFLNNFYPKDINVKWKIDGSERQNGVLNSWTDQDSKDSTYSMSSTLTLTKDEYERHNSYTCEATHKTSTSPIVKSFNRNEC

SEQ ID NO: 23 - protein, 453 aa, Mus musculus
QAQLQQSGAELVRPGASVTLSCKASGYIFTDYEMHWVKQTPVHGLEWIGAIDPETGGTAYNQKFKGKARLTADKSSSTAYMELRSLTSEDSAVYYCTIYYTNHFDYWGQGTTLTVSSAKTTPPSVYPLAPGCGDTTGSSVTLGCLVKGYFPESVTVTWNSGSLSSSVHTFPALLQSGLYTMSSSVTVPSSTWPSQTVTCSVAHPASSTTVDKKLEPSGPISTINPCPPCKECHKCPAPNLEGGPSVFIFPPNIKDVLMISLTPKVTCVVVDVSEDDPDVRISWFVNNVEVHTAQTQTHREDYNSTIRVVSALPIQHQDWMSGKEFKCKVNNKDLPSPIERTISKIKGLVRAPQVYILPPPAEQLSRKDVSLTCLVVGFNPGDISVEWTSNGHTEENYKDTAPVLDSDGSYFIYSKLDIKTSKWEKTDSFSCNVRHEGLKNYYLKKTISRSPGK

SEQ ID NO: 24 - protein, 219 aa, Mus musculus
DVVMTQTPLSLPVSLGDQASISCRSSQSLVYSNGDTYLYWYLQKPGQSPKLLIYKVSNRFSGVPDRFSGSGSGTDFTLKISRVEAEDLGVYFCSQSTHVPLTFGAGTKLELKRADAAPTVSIFPPSSEQLTSGGASVVCFLNNFYPKDINVKWKIDGSERQNGVLNSWTDQDSKDSTYSMSSTLTLTKDEYERHNSYTCEATHKTSTSPIVKSFNRNEC

SEQ ID NO: 25 - protein, 453 aa, Mus musculus
QVQLQQSGAELVRPGASVTLSCKASGYTFTDYEVHWVKQTPVHGLEWIGAIDPETGGTAYNLKFKGKAILTADKSSSTAYMELRSLTSEDSAVYYFTIYYTNNFDYWGQGTALTVSSAKTTPPSVYPLAPGCGDTTGSSVTLGCLVKGYFPESVTVTWNSGSLSSSVHTFPALLQSGLYTMSSSVTVPSSTWPSQTVTCSVAHPASSTTVDKKLEPSGPISTINPCPPCKECHKCPAPNLEGGPSVFIFPPNIKDVLMISLTPKVTCVVVDVSEDDPDVRISWFVNNVEVHTAQTQTHREDYNSTIRVVSALPIQHQDWMSGKEFKCKVNNKDLPSPIERTISKIKGLVRAPQVYILPPPAEQLSRKDVSLTCLVVGFNPGDISVEWTSNGHTEENYKDTAPVLDSDGSYFIYSKLDIKTSKWEKTDSFSCNVRHEGLKNYYLKKTISRSPGK

SEQ ID NO: 26 - protein, 219 aa, Mus musculus
DVVMTQTPLSLPVSLGDQASISCRSSQSLVYSDGNTYLHWYLQKPGQSPKLLIYKVSYRFSGVPDRFSGSGSGTDFTLKISRVEAEDLGVYFCSQSTHVPLTFGAGTKLELKRADAAPTVSIFPPSSEQLTSGGASVVCFLNNFYPKDINVKWKIDGSERQNGVLNSWTDQDSKDSTYSMSSTLTLTKDEYERHNSYTCEATHKTSTSPIVKSFNRNEC